European Patent Application EP 4 613 856 A1, published September 10, 2025. Title: XYLANASE MUTANT HAVING SPECIFIC ACTIVITY. Applicant: QINGDAO VLAND BIOTECH GROUP CO., LTD. The sequence listing filed with the application follows.

SEQUENCE LISTING (4 sequences)

SEQ ID NO: 1 - protein, 225 aa, synthetic construct
QSFCSSASHSGQSVKVTGNKVGTIGGVGYELWADSGNNSATFYSDGSFSCTFQNAGDYLCRSGLSFDSTKTPSQIGRMKADFKLVKQNSSNVGYSYVGVYGWTRSPLVEYYIVDNWLSPFPPGDWVGNKKHGSFTIDGAQYTVYENTRTGPSIDGDTTFNQYFSIRQQARDCGTIDISAHFDQWEKLGMTMGKLHEAKVLGEAGNVNGGASGTADFPYAKVYIGD

SEQ ID NO: 2 - DNA, 684 bp, synthetic construct
  source 1..684: mol_type = other DNA
caaagtttctgtagttcagcttctcactctggacaaagtgtaaaggtaaccggcaacaaggttggaactattggtggtgttggttacgaattatgggctgatagtggtaataacagtgctactttctattctgatggttccttctcatgtactttccaaaatgctggggattacttatgtcgtagtggtctttctttcgatagtactaagaccccatctcaaattggtcgtatgaaggctgatttcaaacttgtcaaacaaaatagttccaatgttggttattcctatgttggtgtttacggttggactagaagtccacttgtcgaatactacattgtcgataattggcttagtccattcccaccaggtgattgggttggtaacaagaagcatggttctttcactattgatggtgctcaatacactgtttatgaaaacactagaactggtccatctattgatggtgataccaccttcaatcaatacttcagtattcgtcaacaagctcgtgattgtggtaccattgatatttctgctcactttgatcaatgggaaaagcttggtatgactatgggtaaattacatgaagccaaggttttaggtgaagccggtaacgttaacggtggtgccagtggtaccgctgatttcccgtacgcaaaggtttacattggtgattaatgataa

SEQ ID NO: 3 - DNA, 34 bp, synthetic construct
  source 1..34: mol_type = other DNA
ggcgaattccaaagtttctgtagttcagcttctc

SEQ ID NO: 4 - DNA, 39 bp, synthetic construct
  source 1..39: mol_type = other DNA
ataggcggccgcttatcattaatcaccaatgtaaacctt